European Patent Specification EP 4 070 112 B1, published March 20, 2024. Title: A neo-epitope specific assay measuring protease mediated degradation of type IV collagen. Applicant: Nordic Bioscience A/S. The sequence listing filed with the application follows.

SEQUENCE LISTING (18 sequences)

SEQ ID NO: 1 - protein, 10 aa, Homo sapiens
MGNTGPTGAV

SEQ ID NO: 2 - protein, 11 aa, Homo sapiens
  VARIANT 1: X = Any amino acid
XMGNTGPTGAV

SEQ ID NO: 3 - protein, 9 aa, Homo sapiens
GNTGPTGAV

SEQ ID NO: 4 - protein, 10 aa, Homo sapiens
MGQTGPTGAV

SEQ ID NO: 5 - protein, 10 aa, Homo sapiens
MGNSGPTGAV

SEQ ID NO: 6 - protein, 10 aa, Homo sapiens
QGNTGPTGAV

SEQ ID NO: 7 - protein, 11 aa, Homo sapiens
FMGNTGPTGAV

SEQ ID NO: 8 - protein, 16 aa, Mus musculus
KSSQSLLYSDGKTYLN

SEQ ID NO: 9 - protein, 7 aa, Mus musculus
LVSKLDS

SEQ ID NO: 10 - protein, 8 aa, Mus musculus
WQGTHFVT

SEQ ID NO: 11 - protein, 7 aa, Mus musculus
TYNIGVG

SEQ ID NO: 12 - protein, 16 aa, Mus musculus
HIWYNDIKYYNTALKS

SEQ ID NO: 13 - protein, 8 aa, Mus musculus
LRPDSFDY

SEQ ID NO: 14 - protein, 78 aa, Mus musculus
KSSQSLLYSDGKTYLNWLLLRPGQSPKRLIYLVSKLDSGVPDRFTGSGSGTDFTLKISRVEAEDLGVYYCWQGTHFVT

SEQ ID NO: 15 - protein, 77 aa, Mus musculus
TYNIGVGWIRQSSGKGLEWLAHIWYNDIKYYNTALKSRLTISKDTSNNQVFLKIASVVTADTATYYCARLRPDSFDY

SEQ ID NO: 16 - protein, 111 aa, Mus musculus
DVVMTQTPLTLSVTIGQPASISCKSSQSLLYSDGKTYLNWLLLRPGQSPKRLIYLVSKLDSGVPDRFTGSGSGTDFTLKISRVEAEDLGVYYCWQGTHFVTFGAGTKLELK

SEQ ID NO: 17 - protein, 118 aa, Mus musculus
QVTLKESGPGILQPSQTLSLTCSFSGFSLTTYNIGVGWIRQSSGKGLEWLAHIWYNDIKYYNTALKSRLTISKDTSNNQVFLKIASVVTADTATYYCARLRPDSFDYWGQGTTLTVSS

SEQ ID NO: 18 - protein, 10 aa, Artificial Sequence
  Nonsense peptide
LLARDFEKNY